European Patent Application EP 4 613 277 A1, published September 10, 2025. Title: 락토바실러스 퍼멘텀 SRK414 균주를 포함하는 인지기능장애 및 알츠하이머병 예방, 개선 또는 치료용 조성물. Applicant: 주식회사 종근당바이오. The sequence listing filed with the application follows.

SEQUENCE LISTING (3 sequences)

SEQ ID NO: 1 - DNA, 1503 bp, Lactobacillus fermentum
  source 1..1503: mol_type = genomic DNA
gctcaggatgaacgccggcggtgtgcctaatacatgcaagtcgaacgcgttggcccaattgattgatggtgcttgcacctgattgattttggtcgccaacgagtggcggacgggtgagtaacacgtaggtaacctgcccagaagcgggggacaacatttggaaacagatgctaataccgcataacaacgttgttcgcatgaacaacgcttaaaagatggcttctcgctatcacttctggatggacctgcggtgcattagcttgttggtggggtaacggcctaccaaggcgatgatgcatagccgagttgagagactgatcggccacaatgggactgagacacggcccatactcctacgggaggcagcagtagggaatcttccacaatgggcgcaagcctgatggagcaacaccgcgtgagtgaagaagggtttcggctcgtaaagctctgttgttaaagaagaacacgtatgagagtaactgttcatacgttgacggtatttaaccagaaagtcacggctaactacgtgccagcagccgcggtaatacgtaggtggcaagcgttatccggatttattgggcgtaaagagagtgcaggcggttttctaagtctgatgtgaaagccttcggcttaaccggagaagtgcatcggaaactggataacttgagtgcagaagagggtagtggaactccatgtgtagcggtggaatgcgtagatatatggaagaacaccagtggcgaaggcggctacctggtctgcaactgacgctgagactcgaaagcatgggtagcgaacaggattagataccctggtagtccatgccgtaaacgatgagtgctaggtgttggagggtttccgcccttcagtgccggagctaacgcattaagcactccgcctggggagtacgaccgcaaggttgaaactcaaaggaattgacgggggcccgcacaagcggtggagcatgtggtttaattcgaagctacgcgaagaaccttaccaggtcttgacatcttgcgccaaccctagagatagggcgtttccttcgggaacgcaatgacaggtggtgcatggtcgtcgtcagctcgtgtcgtgagatgttgggttaagtcccgcaacgagcgcaacccttgttactagttgccagcattaagttgggcactctagtgagactgccggtgacaaaccggaggaaggtggggacgacgtcagatcatcatgccccttatgacctgggctacacacgtgctacaatggacggtacaacgagtcgcgaactcgcgagggcaagcaaatctcttaaaaccgttctcagttcggactgcaggctgcaactcgcctgcacgaagtcggaatcgctagtaatcgcggatcagcatgccgcggtgaatacgttcccgggccttgtacacaccgcccgtcacaccatgagagtttgtaacacccaaagtcggtggggtaaccttttagagccagccgcctaagtgggacagatgattagggtga

SEQ ID NO: 2 - DNA, 17 bp, synthetic construct
  source 1..17: mol_type = other DNA
cctacgggnggcwgcag

SEQ ID NO: 3 - DNA, 21 bp, synthetic construct
  source 1..21: mol_type = other DNA
gactachvgggtatctaatcc